European Patent Specification EP 3 653 048 B9, published October 4, 2023. Title: Methods and Compositions for Targeted Genetic Modification Through Single-Step Multiple Targeting. Applicant: Voronina, Vera Macdonald, Lynn Zambrowicz, Brian Murphy, Andrew J. The sequence listing filed with the application follows.

SEQUENCE LISTING (86 sequences)

SEQ ID NO: 1 - DNA, 23 bp, Artificial Sequence
  a genomic target sequence that is linked to a guide RNA (gRNA)
  misc_feature (2)...(21): n = A,T,C or G
gnnnnnnnnnnnnnnnnnnnngg

SEQ ID NO: 2 - DNA, 42 bp, Artificial Sequence
  ZFN1/2 recognition site
tgcgatcgctgcggccgatcttagccagacgagcgggttcgg

SEQ ID NO: 3 - DNA, 36 bp, Artificial Sequence
  ZFN3/4 recognition site
cgctgcggccgatcttagccagacgagcgggttcgg

SEQ ID NO: 4 - DNA, 39 bp, Artificial Sequence
  ZFN5/6 recognition site
agcgtgtccgacctgatgcagctctcggagggcgaagaa

SEQ ID NO: 5 - DNA, 18 bp, Artificial Sequence
  ZFN1 Binding sequence
tgcgatcgctgcggccga

SEQ ID NO: 6 - DNA, 18 bp, Artificial Sequence
  ZFN2 Binding sequence
ccgaacccgctcgtctgg

SEQ ID NO: 7 - DNA, 15 bp, Artificial Sequence
  ZFN3 Binding sequence
cgctgcggccgatct

SEQ ID NO: 8 - DNA, 15 bp, Artificial Sequence
  ZFN4 Binding sequence
ccgaacccgctcgtc

SEQ ID NO: 9 - DNA, 18 bp, Artificial Sequence
  ZFN5 Binding sequence
agcgtgtccgacctgatg

SEQ ID NO: 10 - DNA, 15 bp, Artificial Sequence
  ZFN6 Binding sequence
ttcttcgccctccga

SEQ ID NO: 11 - DNA, 6 bp, Artificial Sequence
  ZFN1/2 cleavage site
tcttag

SEQ ID NO: 12 - DNA, 6 bp, Artificial Sequence
  ZFN3/4cleavage site
tagcca

SEQ ID NO: 13 - DNA, 6 bp, Artificial Sequence
  ZFN5/6 cleavage site
cagctc

SEQ ID NO: 14 - DNA, 17 bp, Artificial Sequence
  HYG forward primer
tgcggccgatcttagcc

SEQ ID NO: 15 - DNA, 21 bp, Artificial Sequence
  HYG probe
acgagcgggttcggcccattc

SEQ ID NO: 16 - DNA, 18 bp, Artificial Sequence
  HYG reverse primer
ttgaccgattccttgcgg

SEQ ID NO: 17 - DNA, 23 bp, Artificial Sequence
  HYG-U forward primer
cgacgtctgtcgagaagtttctg

SEQ ID NO: 18 - DNA, 24 bp, Artificial Sequence
  HYG-U probe
agttcgacagcgtgtccgacctga

SEQ ID NO: 19 - DNA, 19 bp, Artificial Sequence
  HYG-U reverse primer
cacgccctcctacatcgaa

SEQ ID NO: 20 - DNA, 20 bp, Artificial Sequence
  HYG-D forward primer
tgtcgggcgtacacaaatcg

SEQ ID NO: 21 - DNA, 22 bp, Artificial Sequence
  HYG-D probe
ccgtctggaccgatggctgtgt

SEQ ID NO: 22 - DNA, 20 bp, Artificial Sequence
  HYG-D reverse primer
gggcgtcggtttccactatc

SEQ ID NO: 23 - DNA, 24 bp, Artificial Sequence
  PGKp1 (Hyg Promoter) forward primer
caaatggaagtagcacgtctcact

SEQ ID NO: 24 - DNA, 23 bp, Artificial Sequence
  PGKp1 (Hyg Promoter) probe
ctcgtgcagatggacagcaccgc

SEQ ID NO: 25 - DNA, 15 bp, Artificial Sequence
  PGKp1 (Hyg Promoter) reverse primer
ccgctgccccaaagg

SEQ ID NO: 26 - DNA, 20 bp, Artificial Sequence
  hIgK6 forward primer
gtcaagcactgctggcacac

SEQ ID NO: 27 - DNA, 33 bp, Artificial Sequence
  hIgK6 probe
aacccttgtgctattgaattgctatgctgtcag

SEQ ID NO: 28 - DNA, 20 bp, Artificial Sequence
  hIgK6 reverse primer
tgttgtagaccctccgccac

SEQ ID NO: 29 - DNA, 21 bp, Artificial Sequence
  hIgK12 (MAID 1710 insert) forward primer
ttgcctttctcacacctgcag

SEQ ID NO: 30 - DNA, 25 bp, Artificial Sequence
  hIgK12 (MAID 1710 insert) probe
cagcccatcctgtcacttcgctgga

SEQ ID NO: 31 - DNA, 21 bp, Artificial Sequence
  hIgK12 (MAID 1710 insert) reverse primer
tggcccaacagtacagctcag

SEQ ID NO: 32 - DNA, 22 bp, Artificial Sequence
  hIgK13 forward primer
tcagtcaatcacctttcccagc

SEQ ID NO: 33 - DNA, 28 bp, Artificial Sequence
  hIgK13 probe
tccccaggtagcctcatgaaccaatgtt

SEQ ID NO: 34 - DNA, 23 bp, Artificial Sequence
  hIgK13 reverse primer
cacattactgagtccccacaggg

SEQ ID NO: 35 - DNA, 25 bp, Artificial Sequence
  hIgK14 forward primer
cattgtcaaagaagcactggaaatg

SEQ ID NO: 36 - DNA, 32 bp, Artificial Sequence
  hIgK14 probe
accattgcagtttacccacggttaggattttt

SEQ ID NO: 37 - DNA, 23 bp, Artificial Sequence
  hIgK14 reverse primer
tcttgcaatgggatcatcagatg

SEQ ID NO: 38 - DNA, 19 bp, Artificial Sequence
  Neo forward primer
ggtggagaggctattcggc

SEQ ID NO: 39 - DNA, 23 bp, Artificial Sequence
  Neo probe
tgggcacaacagacaatcggctg

SEQ ID NO: 40 - DNA, 17 bp, Artificial Sequence
  Neo reverse primer
gaacacggcggcatcag

SEQ ID NO: 41 - DNA, 21 bp, Artificial Sequence
  hIgK15 forward primer
caggtgcaaaggtgaccacag

SEQ ID NO: 42 - DNA, 21 bp, Artificial Sequence
  hIgK15 probe
tgggtcctgcccatccatgca

SEQ ID NO: 43 - DNA, 20 bp, Artificial Sequence
  hIgK15 reverse primer
ggcagcctgagtgtcagagc

SEQ ID NO: 44 - DNA, 21 bp, Artificial Sequence
  hIgK25 forward primer
gttcaggccccacagactctc

SEQ ID NO: 45 - DNA, 29 bp, Artificial Sequence
  hIgK25 probe
tcctctctggagcaaccatgaagttccct

SEQ ID NO: 46 - DNA, 19 bp, Artificial Sequence
  hIgK25 reverse primer
cctgaagccatgagggcag

SEQ ID NO: 47 - DNA, 21 bp, Artificial Sequence
  hUbC-D (Neo Promoter) forward primer
agggtaggctctcctgaatcg

SEQ ID NO: 48 - DNA, 20 bp, Artificial Sequence
  hUbC-D (Neo Promoter) probe
acaggcgccggacctctggt

SEQ ID NO: 49 - DNA, 21 bp, Artificial Sequence
  hUbC-D (Neo Promoter) reverse primer
ccaaagaaactgacgcctcac

SEQ ID NO: 50 - DNA, 21 bp, Artificial Sequence
  TCRA Arm4 forward primer
gcgccacatgaatttgaccag

SEQ ID NO: 51 - DNA, 28 bp, Artificial Sequence
  TCRA Arm4 probe
tgtacccaatcttccaaagaaagagctg

SEQ ID NO: 52 - DNA, 19 bp, Artificial Sequence
  TCRA Arm4 reverse primer
ggcatcctgtcctcccttc

SEQ ID NO: 53 - DNA, 27 bp, Artificial Sequence
  Parental 1540m1 forward primer
cagtaagggaagagactacaacagcat

SEQ ID NO: 54 - DNA, 27 bp, Artificial Sequence
  Parental 1540m1 probe
tgcacactgctcaccactgcaagctat

SEQ ID NO: 55 - DNA, 17 bp, Artificial Sequence
  Parental 1540m1 reverse primer
tgctggtggccccatct

SEQ ID NO: 56 - DNA, 28 bp, Artificial Sequence
  Parental 1540m3 forward primer
gaactcagctatgatagtgtcgaatgta

SEQ ID NO: 57 - DNA, 23 bp, Artificial Sequence
  Parental 1540m3 probe
cagcccagcagctgtgggttctc

SEQ ID NO: 58 - DNA, 25 bp, Artificial Sequence
  Parental 1540m3 reverse primer
gctcagggagaacacagaacttaga

SEQ ID NO: 59 - DNA, 20 bp, Artificial Sequence
  hIgK5 forward primer
ccccgtcctcctcctttttc

SEQ ID NO: 60 - DNA, 32 bp, Artificial Sequence
  hIgK5 probe
tcatgtccattaacccatttaccttttgccca

SEQ ID NO: 61 - DNA, 19 bp, Artificial Sequence
  hIgK5 reverse primer
tgcaagtgctgccagcaag

SEQ ID NO: 62 - DNA, 156 bp, Artificial Sequence
  mouse Tcra/5' Frt junction sequence
gtcttttttgttcttcacagttgagcttcatcaaagtcacatgggttaaactctatggagtagtcagaacacactcttcagaagggactcctgatttcaaagggtaccgaagttcctattccgaagttcctattctctagaaagtataggaacttc

SEQ ID NO: 63 - DNA, 132 bp, Artificial Sequence
  3' Frt/human IgK junction sequence
gaagttcctattccgaagttcctattctctagaaagtataggaacttcctagggtttcaccggtggcgcgcctaacagagaggaaagtcaaattataaagaatatgagattcagaattctgattaactgtgg

SEQ ID NO: 64 - DNA, 124 bp, Artificial Sequence
  Human IgK/mouse Tcra junction sequence
gataaattattttgtcagacaacaataaaaatcaatagcacgccctaagagcggccgccaccgcggtggagctcaggtttccggtacttaacaacagagcacagatttagtggtgagggactct

SEQ ID NO: 65 - DNA, 28 bp, Artificial Sequence
  hIgK10 forward primer
cgattatgactggttaggtagaaaggtg

SEQ ID NO: 66 - DNA, 32 bp, Artificial Sequence
  hIgK10 probe
gccactggtttctccaaatgttttcaatccat

SEQ ID NO: 67 - DNA, 24 bp, Artificial Sequence
  hIgK10 reverse primer
gggagtacttggagatccctaagc

SEQ ID NO: 68 - DNA, 136 bp, Artificial Sequence
  mouse Tcra/5' Frt junction sequence
ttgagcttcatcaaagtcacatgggttaaactctatggagtagtcagaacacactcttcagaagggactcctgatttcaaagggtaccgaagttcctattccgaagttcctattctctagaaagtataggaacttc

SEQ ID NO: 69 - DNA, 132 bp, Artificial Sequence
  3' Frt/human IgK junction sequence
gaagttcctattccgaagttcctattctctagaaagtataggaacttcctagggtttcaccggtggcgcgccaggacccaggctctgacactcaggctgccaatacaattgccatgaagacagatgttgatg

SEQ ID NO: 70 - DNA, 23 bp, Artificial Sequence
  gRNA#1 CRISPR recognition sequence
acgagcgggttcggcccattcgg

SEQ ID NO: 71 - DNA, 23 bp, Artificial Sequence
  gRNA#6 CRISPR recognition sequence
cttagccagacgagcgggttcgg

SEQ ID NO: 72 - DNA, 23 bp, Artificial Sequence
  gRNA#10 CRISPR recognition sequence
gccgatcttagccagacgagcgg

SEQ ID NO: 73 - DNA, 23 bp, Artificial Sequence
  gRNA#16 CRISPR recognition sequence
cgacctgatgcagctctcggagg

SEQ ID NO: 74 - DNA, 21 bp, Artificial Sequence
  hIgK22 forward primer
tggctccaagaacagtttgcc

SEQ ID NO: 75 - DNA, 28 bp, Artificial Sequence
  hIgK22 probe
ccctgactttgctgctcaactcacagcc

SEQ ID NO: 76 - DNA, 21 bp, Artificial Sequence
  hIgK22 reverse primer
ggtccagtggaatctgccatg

SEQ ID NO: 77 - DNA, 23 bp, Artificial Sequence
  hIgK21 forward primer
catttggctacatatcaaagccg

SEQ ID NO: 78 - DNA, 27 bp, Artificial Sequence
  hIgK21 probe
cctgagccagggaacagcccactgata

SEQ ID NO: 79 - DNA, 20 bp, Artificial Sequence
  hIgK21 reverse primer
acatggctgaggcagacacc

SEQ ID NO: 80 - DNA, 21 bp, Artificial Sequence
  hIgK26 forward primer
tgggccgttatgctagtacca

SEQ ID NO: 81 - DNA, 25 bp, Artificial Sequence
  hIgK26 probe
tggctttaccccttttgaagggccc

SEQ ID NO: 82 - DNA, 21 bp, Artificial Sequence
  hIgK26 reverse primer
cacagctgaagcaggatgagc

SEQ ID NO: 83 - DNA, 19 bp, Artificial Sequence
  hIgK30 forward primer
tctctgagcagccatcccc

SEQ ID NO: 84 - DNA, 27 bp, Artificial Sequence
  hIgK30 probe
ttctcctttggtgtagagggcaccagc

SEQ ID NO: 85 - DNA, 19 bp, Artificial Sequence
  hIgK30 reverse primer
accaggcatggcagaaagg

SEQ ID NO: 86 - DNA, 130 bp, Artificial Sequence
  3' Frt/human IgK junction
gaagttcctattccgaagttcctattctctagaaagtataggaacttcctagggtttcaccggtggcgcgcctgagtagtgctttaggtgtgtaatcaccaaagatttagtgaagtccctgtgcaaggag